European Patent Application EP 4 194 550 A2, published June 14, 2023. Title: Trichome specific promoters for the manipulation of cannabinoids and other compounds in glandular trichomes. Applicant: 22ND CENTURY LIMITED, LLC. Application EP. The sequence listing filed with the application follows.

SEQUENCE LISTING (33 sequences)

SEQ ID NO: 1 - DNA, 554 bp, synthetic construct
  misc_feature 1..554: note = Description of Artificial Sequence: Synthetic polynucleotide
  source 1..554: mol_type = other DNA
aaaaataaaattaataaatttttaattattaatatcattttattttttaataaataaatatcatttttatattattataatatgtataaagttttaattgtatacaagaagtcttatagtaagagtatacaccttacatcataataactactcgatctgaaatcaatggtcaagaaaagttccctaccggtaggaaacttttgctagatcctaccatagtcttcccttatatttattatgtagaatctattattatatctaataattaacaaatattaacaaatcattttgaaaaattatattaaaaaaaaaacttgaaaagtcaaagattaaccatcaatttgccaaatcaaattagtgagaaagtaggtattatatacctaacactcattttacatatgtctagacgtttatatgtatagcgttgttgtgtgtaataagttcacttgtagtatcttgtacatacataatatatatatataggtgtgtttgtgaacaattatattatcacacatacacaactcattattatcataataataataataccatgg

SEQ ID NO: 2 - DNA, 550 bp, synthetic construct
  misc_feature 1..550: note = Description of Artificial Sequence: Synthetic polynucleotide
  source 1..550: mol_type = other DNA
aaaaataaaattaataaatttttaattattaatatcattttattttttaataaataaatatcatttttatattattataatatgtataaagttttaattgtatacaagaagtcttatagtaagagtatacaccttacatcataataactactcgatctgaaatcaatggtcaagaaaagttccctaccggtaggaaacttttgctagatcctaccatagtcttcccttatatttattatgtagaatctattattatatctaataattaacaaatattaacaaatcattttgaaaaattatattaaaaaaaaaacttgaaaagtcaaagattaaccatcaatttgccaaatcaaattagtgagaaagtaggtattatatacctaacactcattttacatatgtctagacgtttatatgtatagcgttgttgtgtgtaataagttcacttgtagtatcttgtacatacataatatatatatataggtgtgtttgtgaacaattatattatcacacatacacaactcattattatcataataataataataat

SEQ ID NO: 3 - DNA, 558 bp, synthetic construct
  misc_feature 1..558: note = Description of Artificial Sequence: Synthetic polynucleotide
  source 1..558: mol_type = other DNA
aaaaataaaattaataaatttttaattattaatatcattttattttttaataaataaatatcatttttatattattataatatgtataaagttttaattgtatacaagaagtcttatagtaagagtatacaccttacatcataataactactcgatctgaaatcaatggtcaagaaaagttccctaccggtaggaaacttttgctagatcctaccatagtcttcccttatatttattatgtagaatctattattatatctaataattaacaaatattaacaaatcattttgaaaaattatattaaaaaaaaaacttgaaaagtcaaagattaaccatcaatttgccaaatcaaattagtgagaaagtaggtattatatacctaacactcattttacatatgtctagacgtttatatgtatagcgttgttgtgtgtaataagttcacttgtagtatcttgtacatacataatatatatatatataggtgtgtttgtgaacaattatattatcacacatacacaactcattattattagcataataataataataataat

SEQ ID NO: 4 - DNA, 1158 bp, synthetic construct
  misc_feature 1..1158: note = Description of Artificial Sequence: Synthetic polynucleotide
  source 1..1158: mol_type = other DNA
atgaatcatcttcgtgctgagggtccggcctccgttctcgccattggcaccgccaatccggagaacattttattacaagatgagtttcctgactactattttcgcgtcaccaaaagtgaacacatgactcaactcaaagaaaagtttcgaaaaatatgtgacaaaagtatgataaggaaacgtaactgtttcttaaatgaagaacacctaaagcaaaacccaagattggtggagcacgagatgcaaactctggatgcacgtcaagacatgttggtagttgaggttccaaaacttgggaaggatgcttgtgcaaaggccatcaaagaatggggtcaacccaagtctaaaatcactcatttaatcttcactagcgcatcaaccactgacatgcccggtgcagactaccattgcgctaagcttctcggactgagtccctcagtgaagcgtgtgatgatgtatcaactaggctgttatggtggtggaaccgttctacgcattgccaaggacatagcagagaataacaaaggcgcacgagttctcgccgtgtgttgtgacataatggcttgcttgtttcgtgggccttcagagtctgacctcgaattactagtgggacaagctatctttggtgatggggctgctgcggtgattgttggagctgaacccgatgagtcagttggggaaaggccgatatttgagttggtgtcaactgggcaaacaatcttaccaaactcggaaggaactattgggggacatataagggaagcaggactgatatttgatttacataaggatgtgcctatgttgatctctaataatattgagaaatgtttgattgaggcatttactcctattgggattagtgattggaactccatattttggattacacacccaggtgggaaagctattttggacaaagtggaggagaagttgcatctaaagagtgataagtttgtggattcacgtcatgtgctgagtgagcatgggaatatgtctagctcaactgtcttgtttgttatggatgagttgaggaagaggtcgttggaggaagggaagtctaccactggagatggatttgagtggggtgttctttttgggtttggaccaggtttgactgtcgaaagagtggtcgtgcgtagtgttcccatcaaatattaa

SEQ ID NO: 5 - DNA, 996 bp, synthetic construct
  misc_feature 1..996: note = Description of Artificial Sequence: Synthetic polynucleotide
  source 1..996: mol_type = other DNA
aatttttgacaattttttttaatataactaacttgaagataattcctaatacgaataaatacagaaaatataaacagttttgttataacacttttagatcagattataattaaattttatatttttgataaaaaaatcaattgagggtcctatttgtaccattttagaaaatatagtgtccatttttattatttagtaaaacagagagtctaatgcgtaacttttacaaaaatacatggtccaaaatagtatttaccctttaattttattagcaactgtcccaaaaaaaatatgttttgatgactgacgtacgggaatgtaaagttttgtaatagtgtattgattcaaagacaacataaagacatcaatctgaaatcgatttcaatgtcccaaaaacacattaatgagccttaattgcatccgataatcattttccattggttttattacttctcatatatatagacatcacatatatgataggatttcttgagaataatgttaacattgagatttttattacaactgatatattgattatgcttagatggcttgaatttgagcgacatatatagaaagagtatagaatgatatatatgcacatccaaaatatgtaccaaaatattaggtgacaatttagataaatggaagagaaaattatagaaaaatgagggtttatatttttgtggttatttaattttagacatagtgtgatccaataattttaggatgtataattgttaggcacatggattacttgtttttttattaagtataaccttacaaagtagatggtagtaattaatgtagaaggttccaataatgtatttatataaattgttaggcatgcaaagcctaattaattaataaatgagggtggccaatggccactatatatatcaaggcatcgactgtatgtagcataatgtgatttatataattatcaaaaaaaaaaaataaaaataagaagaagaagaaagttgagaaagaccatgg

SEQ ID NO: 6 - DNA, 992 bp, synthetic construct
  misc_feature 1..992: note = Description of Artificial Sequence: Synthetic polynucleotide
  source 1..992: mol_type = other DNA
aatttttgacaattttttttaatataactaacttgaagataattcctaatacgaataaatacagaaaatataaacagttttgttataacacttttagatcagattataattaaattttatatttttgataaaaaaatcaattgagggtcctatttgtaccattttagaaaatatagtgtccatttttattatttagtaaaacagagagtctaatgcgtaacttttacaaaaatacatggtccaaaatagtatttaccctttaattttattagcaactgtcccaaaaaaaatatgttttgatgactgacgtacgggaatgtaaagttttgtaatagtgtattgattcaaagacaacataaagacatcaatctgaaatcgatttcaatgtcccaaaaacacattaatgagccttaattgcatccgataatcattttccattggttttattacttctcatatatatagacatcacatatatgataggatttcttgagaataatgttaacattgagatttttattacaactgatatattgattatgcttagatggcttgaatttgagcgacatatatagaaagagtatagaatgatatatatgcacatccaaaatatgtaccaaaatattaggtgacaatttagataaatggaagagaaaattatagaaaaatgagggtttatatttttgtggttatttaattttagacatagtgtgatccaataattttaggatgtataattgttaggcacatggattacttgtttttttattaagtataaccttacaaagtagatggtagtaattaatgtagaaggttccaataatgtatttatataaattgttaggcatgcaaagcctaattaattaataaatgagggtggccaatggccactatatatatcaaggcatcgactgtatgtagcataatgtgatttatataattatcaaaaaaaaaaaataaaaataagaagaagaagaaagttgagaaagaga

SEQ ID NO: 7 - DNA, 485 bp, synthetic construct
  misc_feature 1..485: note = Description of Artificial Sequence: Synthetic polynucleotide
  source 1..485: mol_type = other DNA
aaaaaagaagaagaagaagaaagttgagaaagagaatggcagtgaagcatttgattgtattgaagttcaaagatgaaatcacagaagcccaaaaggaagaatttttcaagacgtatgtgaatcttgtgaatatcatcccagccatgaaagatgtatactggggtaaagatgtgactcaaaagaataaggaagaagggtacactcacatagttgaggtaacatttgagagtgtggagactattcaggactacattattcatcctgcccatgttggatttggagatgtctatcgttctttctgggaaaaacttctcatttttgactacacaccacgaaagtagactatatatagtagccgaccaagctgccttcatcttcatcttctcaaataatatatctaatatctaattatataataataactacttaataaaagactgtgtttataacattaaataataataataataaagtcttttgtagct

SEQ ID NO: 8 - DNA, 1361 bp, synthetic construct
  misc_feature 1..1361: note = Description of Artificial Sequence: Synthetic polynucleotide
  source 1..1361: mol_type = other DNA
tcaaaccagattttttataataatttacacaccaattaactaagaaattctaactagagttagtgttgaattagaaggagtatcaaggtaacctatctcctttgtctctttaaatttttaaaagaaaagctattgttgtaattagtttggattttatgggttaggttttgtagagtttgtttgagcttaaaattgttgttggtttgatttaaggttgaattctgtgttggtttgtaagattttagctgatgtagttcgtgttggaggagttcgagtttttgaactcaaagtccactcaacaatatggtgaaattagttttaggtggttttagatgcttttgaagtgtatgttttgtttagattaccctctttttggtaagtttgatagcctttggtcaaggaatgacttaattttgaaggtctgaaagttgagtagttttgaactcttttctgcccaaaatggtttcgaatgagttgtacttgtcatatgtgatttgagtggtaaggttcggaagggtagtcctagacagtgttttcaatgattaggtttggggttggtgaatctagagttaagagcctagagttttggttgcttggattggtgtgacctggttgttagtatccttatcaagggatcccgaataggtgatgagtgaggtttggatggtatattctggatcaaaatttttagatggggtccaaactgatagtttcaaaaatgtgtgtgtgtgtctggttaaggatttattttgggaaggctctagttgggaggtcctggattggaagttctagatgtgaggctccgggtaggagggtcctgtaggaagattctagatggtatttggtggtcgagatgagggatttccgaacatgttttaatagttacaataattcataaattttcaacactaaatcaaaatattaattttgatatgattgtataaatttaatctcatcgtagtgtagagctctacatgcatgcatggtttgtatagccataattaattaattaggcaagaaagatagatgtgcctaccatgcatgacttctaaaacatggatgactttaaattttgaaaccaagcaaaaattgttttactataaatcttgttaatttttcattattgatatcactatgttattctaaccctttcgtagccataattagttaattaggcaagaaagatagatgtgcctaccatgcatgacttctaaaacatggatgactttaaattttgaaaccaagcaaaaattattttactataaatcttgttattttttcattattgatatcactatgttattctaaccctttctttccctcattttttcttaatattcaatcaataataatctccatgg

SEQ ID NO: 9 - DNA, 1357 bp, synthetic construct
  misc_feature 1..1357: note = Description of Artificial Sequence: Synthetic polynucleotide
  source 1..1357: mol_type = other DNA
tcaaaccagattttttataataatttacacaccaattaactaagaaattctaactagagttagtgttgaattagaaggagtatcaaggtaacctatctcctttgtctctttaaatttttaaaagaaaagctattgttgtaattagtttggattttatgggttaggttttgtagagtttgtttgagcttaaaattgttgttggtttgatttaaggttgaattctgtgttggtttgtaagattttagctgatgtagttcgtgttggaggagttcgagtttttgaactcaaagtccactcaacaatatggtgaaattagttttaggtggttttagatgcttttgaagtgtatgttttgtttagattaccctctttttggtaagtttgatagcctttggtcaaggaatgacttaattttgaaggtctgaaagttgagtagttttgaactcttttctgcccaaaatggtttcgaatgagttgtacttgtcatatgtgatttgagtggtaaggttcggaagggtagtcctagacagtgttttcaatgattaggtttggggttggtgaatctagagttaagagcctagagttttggttgcttggattggtgtgacctggttgttagtatccttatcaagggatcccgaataggtgatgagtgaggtttggatggtatattctggatcaaaatttttagatggggtccaaactgatagtttcaaaaatgtgtgtgtgtgtctggttaaggatttattttgggaaggctctagttgggaggtcctggattggaagttctagatgtgaggctccgggtaggagggtcctgtaggaagattctagatggtatttggtggtcgagatgagggatttccgaacatgttttaatagttacaataattcataaattttcaacactaaatcaaaatattaattttgatatgattgtataaatttaatctcatcgtagtgtagagctctacatgcatgcatggtttgtatagccataattaattaattaggcaagaaagatagatgtgcctaccatgcatgacttctaaaacatggatgactttaaattttgaaaccaagcaaaaattgttttactataaatcttgttaatttttcattattgatatcactatgttattctaaccctttcgtagccataattagttaattaggcaagaaagatagatgtgcctaccatgcatgacttctaaaacatggatgactttaaattttgaaaccaagcaaaaattattttactataaatcttgttattttttcattattgatatcactatgttattctaaccctttctttccctcattttttcttaatattcaatcaataataatctcc

SEQ ID NO: 10 - DNA, 1188 bp, synthetic construct
  misc_feature 1..1188: note = Description of Artificial Sequence: Synthetic polynucleotide
  source 1..1188: mol_type = other DNA
atgggactctcatcagtttgtaccttttcatttcaaactaattaccatactttattaaatcctcacaataataatcccaaaacctcattattatgttatcgacaccccaaaacaccaattaaatactcttacaataattttccctctaaacattgctccaccaagagttttcatctacaaaacaaatgctcagaatcattatcaatcgcaaaaaattccattagggcagctactacaaatcaaactgagcctccagaatctgataatcattcagtagcaactaaaattttaaactttgggaaggcatgttggaaacttcaaagaccatatacaatcatagcatttacttcatgcgcttgtggattgtttgggaaagagttgttgcataacacaaatttaataagttggtctctgatgttcaaggcattcttttttttggtggctatattatgcattgcttcttttacaactaccatcaatcagatttacgatcttcacattgacagaataaacaagcctgatctaccactagcttcaggggaaatatcagtaaacacagcttggattatgagcataattgtggcactgtttggattgataataactataaaaatgaagggtggaccactctatatatttggctactgttttggtatttttggtgggattgtctattctgttccaccatttagatggaagcaaaatccttccactgcatttcttctcaatttcctggcccatattattacaaatttcacattttattatgccagcagagcagctcttggcctaccatttgagttgaggccttcttttactttcctgctagcatttatgaaatcaatgggttcagctttggctttaatcaaagatgcttcagacgttgaaggcgacactaaatttggcatatcaaccttggcaagtaaatatggttccagaaacttgacattattttgttctggaattgttctcctatcctatgtggctgctatacttgctgggattatctggccccaggctttcaacagtaacgtaatgttactttctcatgcaatcttagcattttggttaatcctccagactcgagattttgcgttaacaaattacgacccggaagcaggcagaagattttacgagttcatgtggaagctttattatgctgaatatttagtatatgttttcatataa

SEQ ID NO: 11 - DNA, 805 bp, synthetic construct
  misc_feature 1..805: note = Description of Artificial Sequence: Synthetic polynucleotide
  source 1..805: mol_type = other DNA
ataatgttatttattatttaatacaatatgacatttatacagcgtaccaaacgagcccataatgtattgcaattgtattgttgtacgaattaaaataataaaatactaattaagttaatattgtaagatagataatatggcaaacaaataaataattttcagttgagaatatgtacaaaattaaagttgattttacaagaaacaagtagtactaattaaaatggtagatttacatatagtgttcgttaaatttgaaaaaagaaaacgactaattcattggaaaattgattgtggaagaaatcaaaatttggtggctgaaccgccctagttacttaacacaattcataaaacaaccctacactacttaccctacactatatacgtatattttttttttatattccatttgttaataaaataaatatgcattgttattatgtgtaccaagatgctaatacggtgacgttttatataagtttataattttttattaaagtaaaacaattgtccctcaatattaaattaaagaaaataagtaggttttagcatttctcatgataaataagtaggagtagtaagtatattaatttatatgcatatgttaaaaggcaacacagtgataggttgtgtagtacgtacccaaaccaaattccagcctaatccattattaatgagcaagtccttgataaaataaggtgcatgttgttagatcaaataacccgtcccgaaatccaatatatatatatatataatattcaaactctctctttctatcttcgtacaatttaatagaagtaaccatggg

SEQ ID NO: 12 - DNA, 800 bp, synthetic construct
  misc_feature 1..800: note = Description of Artificial Sequence: Synthetic polynucleotide
  source 1..800: mol_type = other DNA
ataatgttatttattatttaatacaatatgacatttatacagcgtaccaaacgagcccataatgtattgcaattgtattgttgtacgaattaaaataataaaatactaattaagttaatattgtaagatagataatatggcaaacaaataaataattttcagttgagaatatgtacaaaattaaagttgattttacaagaaacaagtagtactaattaaaatggtagatttacatatagtgttcgttaaatttgaaaaaagaaaacgactaattcattggaaaattgattgtggaagaaatcaaaatttggtggctgaaccgccctagttacttaacacaattcataaaacaaccctacactacttaccctacactatatacgtatattttttttttatattccatttgttaataaaataaatatgcattgttattatgtgtaccaagatgctaatacggtgacgttttatataagtttataattttttattaaagtaaaacaattgtccctcaatattaaattaaagaaaataagtaggttttagcatttctcatgataaataagtaggagtagtaagtatattaatttatatgcatatgttaaaaggcaacacagtgataggttgtgtagtacgtacccaaaccaaattccagcctaatccattattaatgagcaagtccttgataaaataaggtgcatgttgttagatcaaataacccgtcccgaaatccaatatatatatatatataatattcaaactctctctttctatcttcgtacaatttaatagaagtaata

SEQ ID NO: 13 - DNA, 1000 bp, synthetic construct
  misc_feature 1..1000: note = Description of Artificial Sequence: Synthetic polynucleotide
  source 1..1000: mol_type = other DNA
taaaaattagattatatttttatcagaattttttatttatatttttcatcgagttacgttgatttaacgtatgttgacggtgcttataattgtctattatttttaagttatatacacgcactacttacgtaaatttagttggcagattttctgtctctatgggctatattgttggacatcagctatctcattaattaataataccatactttttcttaaaagttaaataaaacaaaattatacacgcactgattcgaatggtgtagcccacgcacttgctaagtctgttactagttctgtaggagttaatgtgtggactgatgcttgtcctagattttatcagctatctcattaattaataataccatactttttcttaaaagttaaataaaacaaaattatacacgcactacgataaggattatataaatgattaactaaaaaatatctatttaacatgccataccgcgaaaggttttgcgccattcgatggtgtccgggatctcgacgctctcccttatgcgactcctgcattaggaagcagcccagtagtaggttgaggccgttgagcaccgccgccgcaaggaatggtgcatgcaaggagatggcgcccaacagtcccccggccacggggcctgccaccatacccacgccgaaacaagcgctcatgagcccgaagtggcgagcccgatcttccccatcggtgatgtcggcgatataggcgccagcaaccgcacctgtggcgccggtgatgccggccacgatgcgtccggcgtagaggatcgagatctcgatcccgcgaaattaatacgactcactataggggaattgtgagcggataacaattcccctctagaaataattttgtttaactttaagaaggagatataccatgaaacaccaccaccaccaccaccaccacggtggtctggttccgcgtggttcccatgatcaaacaagtttgtacaaaaaagcaggctccgaattcgcccttatggag

SEQ ID NO: 14 - DNA, 869 bp, synthetic construct
  misc_feature 1..869: note = Description of Artificial Sequence: Synthetic polynucleotide
  source 1..869: mol_type = other DNA
gtgacaaactgaagaattctgtttattttattttatacattagtgatgttttttacttttttagagttatttttatgcctatgtaatttgcatattgtagtggagtttatgcagttatttttttgttgttatttagttgtttaactaagagaaataaatatatatattttttatttgtgcgttgtttttattttattttttaagttgacgtaagtgttgatgctcaattaatttttatattaacataaaattgttattgtgttgcttattcgttgctattgagttatttcaatattgtactttttgaagtttttgtcttataaatttatttttatttgcataacatatgataaactttaatggatttatatgttacggttaagttgttttctagttgcttttgtgttgttgtttagttgttttgcgctgagaaaagaagccctatacgttaaaattcactttgtccgaattcgccacgtggcaactactgctacgttctgacgctacagattgtgagcgtcaggcaagtctgaatgctttgtcccgcactcacgtgtgagtctcactcgcccacatagccatatgtgtgccacacatctccttgcgcatctaggggagtttttctactgtatttttgtaaataagaaactttgaaaatagtatatttgaaattaataaataatataaatgtttatttttacttatagtagtataaatatttatttaagataattttaacttaaaatagaaaaaatctcaaaaaaaaataaaataaaataaactatacctttaatttttatatttatgaaaatttcccgtataaaagggaagatttttttttttaaaattagtaggtaagtaataggatg

SEQ ID NO: 15 - DNA, 2351 bp, synthetic construct
  misc_feature 1..2351: note = Description of Artificial Sequence: Synthetic polynucleotide
  source 1..2351: mol_type = other DNA
tcttggagtgtatatatagatatatatatacatttctccatttttggccacccaaattacctaaattgaattcgtcgtgttcgtctttctccgccataaataacaattgatttccttcgttctttcaagtttttgtcaactgagtactgagatccagtctgagtcgacacttgtagaggttcgaaaatggcgcagaagaagtttatttttgaggttgaaaaggctaaggaagctaaggatggaaggccttccatgggacctgtttatcgaagtatgtacgccaaggatggctttcctcctccgattgatggattggattgttgttgggatgtgtttaggctttctgtggagagaaatcctggaaacaaaatgctcggtcgccgggaggttgtggatgggaaggctggaaagtatgtttggcaaacttataaggaggtttatgattgtgtgataaaacttggaaatgccatgcgcagttgtggtttcggagaaggagacaaatgtggtatctatggtgccaattgctctgaatggattatgagcatgcaggcttgcaatgctcatggactctattgtgttccgttgtatgacaccttaggtgctaatgcaattgagtttgtcataaaacatgccgaggttacaattgcttttgcagaagagaaaaagcttcctgagctgttgaaaacacttcctaacaccacagactatttaaaaacacttgtgagctttgggaaggtcacaccggaacaaagggaatctgttgaaaagtttggattgaagatctattcctgggaagagttcttgcaattgggtgattgtaaagatttcgatcttccagtgaaaaagaaaactgatatatgcactataatgtatactagtggaactactggtgacccaaagggagtactgatatccaatgagagcatcatttctcttttggctggggtgaggcgattgcttgagagtgtaaatgaaaagttgaccgagaaagatgtatttctttcatatcttccccttgcacatatcttcgatcgggtgattgaggagttatttattttgcatggtgcctcaatcgggttctggcgtggcgatgtcaaattattacttgaagacattggggagctaaaaccaactattttctgtgccgttccccgtgtgctggatagagtctatgctggtttgacgcagaagatttctgctgggggattcttaaagaagactctcttcaatttcgcatactcacgcaagtataataacatgcgaaaggggcttaaacacggggacgcagctccattatgtgacaaaattgtatttagtaaggtgaagcaaggtttgggaggtaatgtgcggcttattctgtctggagctgcgcctctagctcctcatgttgaagcttacttacgagttgtgacatgtgctcatgtttgccaaggatatgggctaactgaaacttgtgcggggacatttgtctcgataccaaatgaactaccaatgctcggtacagttggtcctccagtacccaatgttgatgtatgtctggaatcagttccggaaatgggatatgatgcccttgcagaagtaccgcgtggagaagtatgtgtgaagggaagcaccttattctctgggtactacaaacgtgaagacttaaccaaggaggtcatgattgatgggtggttccatacaggtgatgttggtgagtggcaagcagatggaagcttgaaaatcattgaccgtaagaaaaatattttcaaactttctcaaggagaatatgtggcagttgagaacttagagaacatttatggtcttgtttctgacattgactcaatatgggtttacgggaacagcttcgagtccttcctcgttgctgtgattaacccgaaccagcaagcacttgaacgttgggccggagagaataatatatctggtgacttcaagtccatttgtgaaaatccaagagcaaaggaatacattttgggagagctcaataagattggcaaagagaaaaagttgaaaggttttgagttcataagagctgttcaccttgacccagaggcatttgacatagaacgtgaccttattactccaacatataagaaaaagagaccccagttgctcaaatactaccagagtgttattgataacatgtacaaggaaggaaacaagcccaggacctgaaagatataatagacatttagagcttcactttctaatatttcttcacacacttcccattttcatctctctcttacttattacactataaataattaacaaggtttactgtgttgtaaatgacattttaatattttcatagtctcaatgtttcaattcttagaggacgttttgattgg

SEQ ID NO: 16 - DNA, 420 bp, synthetic construct
  misc_feature 1..420: note = Description of Artificial Sequence: Synthetic polynucleotide
  source 1..420: mol_type = other DNA
gttaataaacatacttgtgagtagatctaagatcctggtaaaataattcccaacatatttcaatcgtaaattcatgagtgattcttatcacttcttaaaaaaaagatataaagatccatagataaatatttgctagtcctttctttccatagtcaacttcaatatggcatcttaacttctttccatcaacaaatgatgctcaactacttaatgtacaatttatatttatttttagtaagggatacacctaacaatgatgcctaattttggtgaatttttttttaccacatgtgacttaatgatatcaaatttggaaatatttagttaatttatttgcccctgctccattatataaagctataaataggatagttcttaattcatagtaattcaaaaattattagaactaaagaaccatgg

SEQ ID NO: 17 - DNA, 416 bp, synthetic construct
  misc_feature 1..416: note = Description of Artificial Sequence: Synthetic polynucleotide
  source 1..416: mol_type = other DNA
gttaataaacatacttgtgagtagatctaagatcctggtaaaataattcccaacatatttcaatcgtaaattcatgagtgattcttatcacttcttaaaaaaaagatataaagatccatagataaatatttgctagtcctttctttccatagtcaacttcaatatggcatcttaacttctttccatcaacaaatgatgctcaactacttaatgtacaatttatatttatttttagtaagggatacacctaacaatgatgcctaattttggtgaatttttttttaccacatgtgacttaatgatatcaaatttggaaatatttagttaatttatttgcccctgctccattatataaagctataaataggatagttcttaattcatagtaattcaaaaattattagaactaaagaaaa

SEQ ID NO: 18 - DNA, 535 bp, synthetic construct
  misc_feature 1..535: note = Description of Artificial Sequence: Synthetic polynucleotide
  source 1..535: mol_type = other DNA
agacgttatagctttattgtctaaatttcttggggtagttttgtcccatgttgctcgcttactttagaagttcaaagtttgacaaaacatgctattcggttatacaatgagctatcctagttcaaggagattcctgtgctatttgtggatgtctacattgtaaattcatgagtgattcttataactttattaaaaaaaagacaaatagatccatagataaatatttgcaagtgctttcttgtcatagcaatttttttttacataggtaatttaaaaaattcatcttaactttttttcatcaataaatgatgctcaattattcaatgcaccatgtacatttatttttaataagggctgcacctaacaaaggtgcctaattttggtaaaaaagaaattacggcatgtgaatatttaatgagcatcaaattacaaaatatttagctaatttctttacccccactccaatctataaagctataaataggataattttccattcatagtaatttccaacattacgactaaagaaccatgg

SEQ ID NO: 19 - DNA, 531 bp, synthetic construct
  misc_feature 1..531: note = Description of Artificial Sequence: Synthetic polynucleotide
  source 1..531: mol_type = other DNA
agacgttatagctttattgtctaaatttcttggggtagttttgtcccatgttgctcgcttactttagaagttcaaagtttgacaaaacatgctattcggttatacaatgagctatcctagttcaaggagattcctgtgctatttgtggatgtctacattgtaaattcatgagtgattcttataactttattaaaaaaaagacaaatagatccatagataaatatttgcaagtgctttcttgtcatagcaatttttttttacataggtaatttaaaaaattcatcttaactttttttcatcaataaatgatgctcaattattcaatgcaccatgtacatttatttttaataagggctgcacctaacaaaggtgcctaattttggtaaaaaagaaattacggcatgtgaatatttaatgagcatcaaattacaaaatatttagctaatttctttacccccactccaatctataaagctataaataggataattttccattcatagtaatttccaacattacgactaaagaaaa

SEQ ID NO: 20 - DNA, 1635 bp, synthetic construct
  misc_feature 1..1635: note = Description of Artificial Sequence: Synthetic polynucleotide
  source 1..1635: mol_type = other DNA
atgaagtgctcaacattctccttttggtttgtttgcaagataatatttttctttttctcattcaatatccaaacttccattgctaatcctcgagaaaacttccttaaatgcttctcgcaatatattcccaataatgcaacaaatctaaaactcgtatacactcaaaacaacccattgtatatgtctgtcctaaattcgacaatacacaatcttagattcacctctgacacaaccccaaaaccacttgttatcgtcactccttcacatgtctctcatatccaaggcactattctatgctccaagaaagttggcttgcagattcgaactcgaagtggtggtcatgattctgagggcatgtcctacatatctcaagtcccatttgttatagtagacttgagaaacatgcgttcaatcaaaatagatgttcatagccaaactgcatgggttgaagccggagctacccttggagaagtttattattgggttaatgagaaaaatgagaatcttagtttggcggctgggtattgccctactgtttgcgcaggtggacactttggtggaggaggctatggaccattgatgagaaactatggcctcgcggctgataatatcattgatgcacacttagtcaacgttcatggaaaagtgctagatcgaaaatctatgggggaagatctcttttgggctttacgtggtggtggagcagaaagcttcggaatcattgtagcatggaaaattagactggttgctgtcccaaagtctactatgtttagtgttaaaaagatcatggagatacatgagcttgtcaagttagttaacaaatggcaaaatattgcttacaagtatgacaaagatttattactcatgactcacttcataactaggaacattacagataatcaagggaagaataagacagcaatacacacttacttctcttcagttttccttggtggagtggatagtctagtcgacttgatgaacaagagttttcctgagttgggtattaaaaaaacggattgcagacaattgagctggattgatactatcatcttctatagtggtgttgtaaattacgacactgataattttaacaaggaaattttgcttgatagatccgctgggcagaacggtgctttcaagattaagttagactacgttaagaaaccaattccagaatctgtatttgtccaaattttggaaaaattatatgaagaagatataggagctgggatgtatgcgttgtacccttacggtggtataatggatgagatttcagaatcagcaattccattccctcatcgagctggaatcttgtatgagttatggtacatatgtagttgggagaagcaagaagataacgaaaagcatctaaactggattagaaatatttataacttcatgactccttatgtgtccaaaaatccaagattggcatatctcaattatagagaccttgatataggaataaatgatcccaagaatccaaataattacacacaagcacgtatttggggtgagaagtattttggtaaaaattttgacaggctagtaaaagtgaaaaccctggttgatcccaataacttttttagaaacgaacaaagcatcccacctcttccacggcatcgtcattaa

SEQ ID NO: 21 - DNA, 800 bp, synthetic construct
  misc_feature 1..800: note = Description of Artificial Sequence: Synthetic polynucleotide
  source 1..800: mol_type = other DNA
cttatcactcattcgggagcaacttaaaaaaattacaattattatgaaagacggcacaaaaagcgaattaattacctaatcgtaaataaaagaaattttacataaatatattatataattttatattattcataaaaaatataaaatagtattagactgaattgagatttgattcgtaactaaaaattaatttctttaatgtaaaattttaaaaacaaattattaaaaccgcgtgaagcgcggatctattccctagttgaataataaagtagatagtagaggaggttagaatttataatttttcatttaaatatttgaatttactttactgttctttgttattcttcatttaattttgctatttgttattttacttttcaaaaattataattttaattaccaaataaaaagtaaaatagatattggtacttgatattcactctttatgggaaccataataaactataaaagtcattatgtgtacttgctaccataggcacctatatcccacaaactagctaccatagccaatttcttgttttttgtttccaatatccaatttttattgatgccaaactattcaatgtacaatgtacatttattttcaataagggcttcacctaacaaaggtgcctaattttagttgatttattttttatcacatgtgactatttaatgactatcaaattataaaatatttaagtcaatttatttgccccaactccaatatataatattataaataggatagttctcaattcctaataattcaaaaaatcattaggactgaagaaccatgg

SEQ ID NO: 22 - DNA, 796 bp, synthetic construct
  misc_feature 1..796: note = Description of Artificial Sequence: Synthetic polynucleotide
  source 1..796: mol_type = other DNA
cttatcactcattcgggagcaacttaaaaaaattacaattattatgaaagacggcacaaaaagcgaattaattacctaatcgtaaataaaagaaattttacataaatatattatataattttatattattcataaaaaatataaaatagtattagactgaattgagatttgattcgtaactaaaaattaatttctttaatgtaaaattttaaaaacaaattattaaaaccgcgtgaagcgcggatctattccctagttgaataataaagtagatagtagaggaggttagaatttataatttttcatttaaatatttgaatttactttactgttctttgttattcttcatttaattttgctatttgttattttacttttcaaaaattataattttaattaccaaataaaaagtaaaatagatattggtacttgatattcactctttatgggaaccataataaactataaaagtcattatgtgtacttgctaccataggcacctatatcccacaaactagctaccatagccaatttcttgttttttgtttccaatatccaatttttattgatgccaaactattcaatgtacaatgtacatttattttcaataagggcttcacctaacaaaggtgcctaattttagttgatttattttttatcacatgtgactatttaatgactatcaaattataaaatatttaagtcaatttatttgccccaactccaatatataatattataaataggatagttctcaattcctaataattcaaaaaatcattaggactgaagaaaa

SEQ ID NO: 23 - DNA, 796 bp, synthetic construct
  misc_feature 1..796: note = Description of Artificial Sequence: Synthetic polynucleotide
  source 1..796: mol_type = other DNA
ttatttaaatttctcagagagatatagagaatttacaataggtcaagttgtatattttttaatccgaataattaatgcttttgaatatccatcatcaatattgaataataaagtagatagcagaggagattagaactcataatttttcatttatatttttgaatttagtttactgttctttattattcttcatttaattttgctatatgttattttacttttcaaaaattctaattttgattaccaaataaaaaataaaatatatattggtacttcatatttagtttttatgggaatgataatgaatgatattgtaataaactataaaagtaattttgtatacttgcatagttcttaatttttacccaaaaaaatatatattaatgaaaaaaaaaggtggaaagtgccataggcacctatatcccacaaactagctataagatattgaaagacaaatagatccatagataaatatttgcgtgtcctttcttttcatatctaattttttgtttttttatttttttccaatagtcaattttggcagcttaacttctttccataaataatgatgccaaactattcaatgtaaaatttagatttattttcattaagggcttcacctaacaaatgtgcctaatttttgtggatttttttaccatatgtcgctatttaatgactaccaaattatagaattatttaagtcaatttctcagtccccgctccaatatataaagttatagaaaggacaattcttaattcatagtaattcaaaaatcattaagactaaaaaccatgg

SEQ ID NO: 24 - DNA, 792 bp, synthetic construct
  misc_feature 1..792: note = Description of Artificial Sequence: Synthetic polynucleotide
  source 1..792: mol_type = other DNA
ttatttaaatttctcagagagatatagagaatttacaataggtcaagttgtatattttttaatccgaataattaatgcttttgaatatccatcatcaatattgaataataaagtagatagcagaggagattagaactcataatttttcatttatatttttgaatttagtttactgttctttattattcttcatttaattttgctatatgttattttacttttcaaaaattctaattttgattaccaaataaaaaataaaatatatattggtacttcatatttagtttttatgggaatgataatgaatgatattgtaataaactataaaagtaattttgtatacttgcatagttcttaatttttacccaaaaaaatatatattaatgaaaaaaaaaggtggaaagtgccataggcacctatatcccacaaactagctataagatattgaaagacaaatagatccatagataaatatttgcgtgtcctttcttttcatatctaattttttgtttttttatttttttccaatagtcaattttggcagcttaacttctttccataaataatgatgccaaactattcaatgtaaaatttagatttattttcattaagggcttcacctaacaaatgtgcctaatttttgtggatttttttaccatatgtcgctatttaatgactaccaaattatagaattatttaagtcaatttctcagtccccgctccaatatataaagttatagaaaggacaattcttaattcatagtaattcaaaaatcattaagactaaaaaaa

SEQ ID NO: 25 - DNA, 720 bp, synthetic construct
  misc_feature 1..720: note = Description of Artificial Sequence: Synthetic polynucleotide
  source 1..720: mol_type = other DNA
ttttcaattgatttaatttcttatattgatataaagaatttgcaatacattgagtttcttaacccgaatattaaacggttttgaatatcttcatcattgattgaataataaagtggatagtagagggaattagaatccataattttttatttatatatttgaagttagtttattattctttgctatccttcatttaattttgctatttgttattttagtttcaaaaatttatttttcattacaaaataaaaaataagataggatattggtacttgataagtcttctttgtggaaacgataatcggtattattaggtatatttgcatatttcaatattattgcaaaaaataaatatattaataaataaagtggaaggtgccataggtacctatatccacaaactagcatattgaaagaaaatggatccaaggataaatatttgcaagtctttttttttttgcatagccaatttctttttttattattattttaatagaatatttcaaaagggcatctaacatttatttttaataaggactgcacctaacaaaggtgcctaatttttgtgaacttttttttaccacatgtgactatttaatgagtactaaattatgaaatatttagttaatttctttgcccccgctccaatatataatgctataaatagcataattttctattcatagtaattcaaaaatcattaggactaaagaaccatgg

SEQ ID NO: 26 - DNA, 716 bp, synthetic construct
  misc_feature 1..716: note = Description of Artificial Sequence: Synthetic polynucleotide
  source 1..716: mol_type = other DNA
ttttcaattgatttaatttcttatattgatataaagaatttgcaatacattgagtttcttaacccgaatattaaacggttttgaatatcttcatcattgattgaataataaagtggatagtagagggaattagaatccataattttttatttatatatttgaagttagtttattattctttgctatccttcatttaattttgctatttgttattttagtttcaaaaatttatttttcattacaaaataaaaaataagataggatattggtacttgataagtcttctttgtggaaacgataatcggtattattaggtatatttgcatatttcaatattattgcaaaaaataaatatattaataaataaagtggaaggtgccataggtacctatatccacaaactagcatattgaaagaaaatggatccaaggataaatatttgcaagtctttttttttttgcatagccaatttctttttttattattattttaatagaatatttcaaaagggcatctaacatttatttttaataaggactgcacctaacaaaggtgcctaatttttgtgaacttttttttaccacatgtgactatttaatgagtactaaattatgaaatatttagttaatttctttgcccccgctccaatatataatgctataaatagcataattttctattcatagtaattcaaaaatcattaggactaaagaaag

SEQ ID NO: 27 - DNA, 1635 bp, synthetic construct
  misc_feature 1..1635: note = Description of Artificial Sequence: Synthetic polynucleotide
  source 1..1635: mol_type = other DNA
atgaattgctcagcattttccttttggtttgtttgcaaaataatatttttctttctctcattcaatatccaaatttcaatagctaatcctcaagaaaacttccttaaatgcttctcggaatatattcctaacaatccagcaaatccaaaattcatatacactcaacacgaccaattgtatatgtctgtcctgaattcgacaatacaaaatcttagattcacctctgatacaaccccaaaaccactcgttattgtcactccttcaaatgtctcccatatccaggccagtattctctgctccaagaaagttggtttgcagattcgaactcgaagcggtggccatgatgctgagggtatgtcctacatatctcaagtcccatttgttgtagtagacttgagaaacatgcattcgatcaaaatagatgttcatagccaaactgcgtgggttgaagccggagctacccttggagaagtttattattggatcaatgagaagaatgagaattttagttttcctggtgggtattgccctactgttggcgtaggtggacactttagtggaggaggctatggagcattgatgcgaaattatggccttgcggctgataatatcattgatgcacacttagtcaatgttgatggaaaagttctagatcgaaaatccatgggagaagatctattttgggctatacgtggtggaggaggagaaaactttggaatcattgcagcatggaaaatcaaactggttgttgtcccatcaaagtctactatattcagtgttaaaaagaacatggagatacatgggcttgtcaagttatttaacaaatggcaaaatattgcttacaagtatgacaaagatttagtactcatgactcacttcataacaaagaatattacagataatcatgggaagaataagactacagtacatggttacttctcttcaatttttcatggtggagtggatagtctagtcgacttgatgaacaagagctttcctgagttgggtattaaaaaaactgattgcaaagaatttagctggattgatacaaccatcttctacagtggtgttgtaaattttaacactgctaattttaaaaaggaaattttgcttgatagatcagctgggaagaagacggctttctcaattaagttagactatgttaagaaaccaattccagaaactgcaatggtcaaaattttggaaaaattatatgaagaagatgtaggagctgggatgtatgtgttgtacccttacggtggtataatggaggagatttcagaatcagcaattccattccctcatcgagctggaataatgtatgaactttggtacactgcttcctgggagaagcaagaagataatgaaaagcatataaactgggttcgaagtgtttataattttacgactccttatgtgtcccaaaatccaagattggcgtatctcaattatagggaccttgatttaggaaaaactaatcctgagagtcctaataattacacacaagcacgtatttggggtgaaaagtattttggtaaaaattttaacaggttagttaaggtgaaaaccaaagctgatcccaataatttttttagaaacgaacaaagtatcccacctcttccaccgcatcatcat

SEQ ID NO: 28 - DNA, 804 bp, synthetic construct
  misc_feature 1..804: note = Description of Artificial Sequence: Synthetic polynucleotide
  source 1..804: mol_type = other DNA
gataatttttcttccaaatttaatagtatcttttatataagttcagtcatgtttttcttatgtaagttaggctattaattattttgatgtatttattatattgtatgtcgtttactgcattctgccaacattggtttttgtcgatttatgatatataatatgatatgctgttaagttagaggtaagattcaatttatttaagattatttaatttgcgcttttattatatacatcttctagttgtaattaatggggtagaattaagactgtgttttgaattaatatcggtattagaataggatttgcatgactatatttctaccttaccaagttttttatctgataacaccctttcacttattattttcttatttttaatttatttatatttttaccatattctatttatactaatcttaagtggtacattacctccctgtggatacgacatataatctgtttactatcgtgaccgaagtataactaattgggcgacatcacacctatatcccacaaactagctactatagtcaatttcttgttttttttccaatagccaattttaaatgatgccaaactattcaatgtataatgtacatttattttaaataagggcttcacctaacaaatgtgcctaattttagttaatttatttttttatcgcatcttactatttaaaggaactatcaaattataaaatatttatgtcaattcatttgccccaactccaatatataatattataaataggatagttctctattcataataattcaaaatatcattaggactgaagaaccatgg

SEQ ID NO: 29 - DNA, 800 bp, synthetic construct
  misc_feature 1..800: note = Description of Artificial Sequence: Synthetic polynucleotide
  source 1..800: mol_type = other DNA
gataatttttcttccaaatttaatagtatcttttatataagttcagtcatgtttttcttatgtaagttaggctattaattattttgatgtatttattatattgtatgtcgtttactgcattctgccaacattggtttttgtcgatttatgatatataatatgatatgctgttaagttagaggtaagattcaatttatttaagattatttaatttgcgcttttattatatacatcttctagttgtaattaatggggtagaattaagactgtgttttgaattaatatcggtattagaataggatttgcatgactatatttctaccttaccaagttttttatctgataacaccctttcacttattattttcttatttttaatttatttatatttttaccatattctatttatactaatcttaagtggtacattacctccctgtggatacgacatataatctgtttactatcgtgaccgaagtataactaattgggcgacatcacacctatatcccacaaactagctactatagtcaatttcttgttttttttccaatagccaattttaaatgatgccaaactattcaatgtataatgtacatttattttaaataagggcttcacctaacaaatgtgcctaattttagttaatttatttttttatcgcatcttactatttaaaggaactatcaaattataaaatatttatgtcaattcatttgccccaactccaatatataatattataaataggatagttctctattcataataattcaaaatatcattaggactgaagaaaa

SEQ ID NO: 30 - DNA, 1635 bp, synthetic construct
  misc_feature 1..1635: note = Description of Artificial Sequence: Synthetic polynucleotide
  source 1..1635: mol_type = other DNA
atgaattgctcaacattctccttttggtttgtttgcaaaataatatttttctttctctcattcaatatccaaatttcaatagctaatcctcaagaaaacttccttaaatgcttctcggaatatattcctaacaatccagcaaatccaaaattcatatacactcaacacgaccaattgtatatgtctgtcctgaattcgacaatacaaaatcttagattcacctctgatacaaccccaaaaccactcgttattgtcactccttcaaatgtctcccatatccaggccagtattctctgctccaagaaagttggtttgcagattcgaactcgaagcggtggccatgatgctgagggtttgtcctacatatctcaagtcccatttgctatagtagacttgagaaacatgcatacggtcaaagtagatattcatagccaaactgcgtgggttgaagccggagctacccttggagaagtttattattggatcaatgagatgaatgagaattttagttttcctggtgggtattgccctactgttggcgtaggtggacactttagtggaggaggctatggagcattgatgcgaaattatggccttgcggctgataatatcattgatgcacacttagtcaatgttgatggaaaagttctagatcgaaaatccatgggagaagatctattttgggctatacgtggtggaggaggagaaaactttggaatcattgcagcatgtaaaatcaaacttgttgttgtcccatcaaaggctactatattcagtgttaaaaagaacatggagatacatgggcttgtcaagttatttaacaaatggcaaaatattgcttacaagtatgacaaagatttaatgctcacgactcacttcagaactaggaatattacagataatcatgggaagaataagactacagtacatggttacttctcttccatttttcttggtggagtggatagtctagttgacttgatgaacaagagctttcctgagttgggtattaaaaaaactgattgcaaagaattgagctggattgatacaaccatcttctacagtggtgttgtaaattacaacactgctaattttaaaaaggaaattttgcttgatagatcagctgggaagaagacggctttctcaattaagttagactatgttaagaaactaatacctgaaactgcaatggtcaaaattttggaaaaattatatgaagaagaggtaggagttgggatgtatgtgttgtacccttacggtggtataatggatgagatttcagaatcagcaattccattccctcatcgagctggaataatgtatgaactttggtacactgctacctgggagaagcaagaagataacgaaaagcatataaactgggttcgaagtgtttataatttcacaactccttatgtgtcccaaaatccaagattggcgtatctcaattatagggaccttgatttaggaaaaactaatcctgagagtcctaataattacacacaagcacgtatttggggtgaaaagtattttggtaaaaattttaacaggttagttaaggtgaaaaccaaagctgatcccaataatttttttagaaacgaacaaagtatcccacctcttccaccgcgtcatcat

SEQ ID NO: 31 - DNA, 171 bp, synthetic construct
  misc_feature 1..171: note = Description of Artificial Sequence: Synthetic polynucleotide
  source 1..171: mol_type = other DNA
atgatgccaaactattcaatgtacaatgtacatttatttttaataagggcttcacctaacaaaggtgcctaatttttgtgaacttttttttaccacatgtgactatttaatgactatcaaattataaaatatttaagtcaatttctttgcccccactccaatatataatgt

SEQ ID NO: 32 - DNA, 232 bp, synthetic construct
  misc_feature 1..232: note = Description of Artificial Sequence: Synthetic polynucleotide
  source 1..232: mol_type = other DNA
atgatgccaaactattcaatgtacaatgtacatttatttttaataagggcttcacctaacaaaggtgcctaatttttgtgaacttttttttaccacatgtgactatttaatgactatcaaattataaaatatttaagtcaatttctttgcccccactccaatatataatgttataaataggataattctcaattcatagtaattcaaaaatcattaggactaaagaaaaatg

SEQ ID NO: 33 - DNA, 709 bp, synthetic construct
  misc_feature 1..709: note = Description of Artificial Sequence: Synthetic polynucleotide
  source 1..709: mol_type = other DNA
atgatgccaaactattcaatgtacaatgtacatttatttttaataagggcttcacctaacaaaggtgcctaatttttgtgaacttttttttaccacatgtgactatttaatgactatcaaattataaaatatttaagtcaatttctttgcccccactccatgatgccaaactattcaatgtacaatgtacatttatttttaataagggcttcacctaacaaaggtgcctaatttttgtgaacttttttttaccacatgtgactatttaatgactatcaaattataaaatatttaagtcaatttctttgcccccactccatgatgccaaactattcaatgtacaatgtacatttatttttaataagggcttcacctaacaaaggtgcctaatttttgtgaacttttttttaccacatgtgactatttaatgactatcaaattataaaatatttaagtcaatttctttgcccccactccatgatgccaaactattcaatgtacaatgtacatttatttttaataagggcttcacctaacaaaggtgcctaatttttgtgaacttttttttaccacatgtgactatttaatgactatcaaattataaaatatttaagtcaatttctttgcccccactccaatatataatgttataaataggataattctcaattcatagtaattcaaaaatcattaggactaaagaaaaatg